European Patent Application EP 4 124 658 A2, published February 1, 2023. Title: TREATMENT OF AMYOTROPHIC LATERAL SCLEROSIS (ALS). Applicant: VOYAGER THERAPEUTICS, INC. THE CURATORS OF THE UNIVERSITY OF MISSOURI. Application PCT/USXXXX/XXXXXX. The sequence listing filed with the application follows.

SEQUENCE LISTING (147 sequences)

SEQ ID NO: 1 - DNA, 981 bp, Homo sapiens
gtttggggccagagtgggcgaggcgcggaggtctggcctataaagtagtcgcggagacggggtgctggtttgcgtcgtagtctcctgcagcgtctggggtttccgttgcagtcctcggaaccaggacctcggcgtggcctagcgagttatggcgacgaaggccgtgtgcgtgctgaagggcgacggcccagtgcagggcatcatcaatttcgagcagaaggaaagtaatggaccagtgaaggtgtggggaagcattaaaggactgactgaaggcctgcatggattccatgttcatgagtttggagataatacagcaggctgtaccagtgcaggtcctcactttaatcctctatccagaaaacacggtgggccaaaggatgaagagaggcatgttggagacttgggcaatgtgactgctgacaaagatggtgtggccgatgtgtctattgaagattctgtgatctcactctcaggagaccattgcatcattggccgcacactggtggtccatgaaaaagcagatgacttgggcaaaggtggaaatgaagaaagtacaaagacaggaaacgctggaagtcgtttggcttgtggtgtaattgggatcgcccaataaacattcccttggatgtagtctgaggccccttaactcatctgttatcctgctagctgtagaaatgtatcctgataaacattaaacactgtaatcttaaaagtgtaattgtgtgactttttcagagttgctttaaagtacctgtagtgagaaactgatttatgatcacttggaagatttgtatagttttataaaactcagttaaaatgtctgtttcaatgacctgtattttgccagacttaaatcacagatgggtattaaacttgtcagaatttctttgtcattcaagcctgtgaataaaaaccctgtatggcacttattatgaggctattaaaagaatccaaattcaaactaaaaaaaaaaaaaaaaaa

SEQ ID NO: 2 - DNA, 465 bp, Macaca fascicularis
atggcgatgaaggccgtgtgcgtgttgaagggcgacagcccagtgcagggcaccatcaatttcgagcagaaggaaagtaatggaccagtgaaggtgtggggaagcattacaggattgactgaaggcctgcatggattccatgttcatcagtttggagataatacacaaggctgtaccagtgcaggtcctcactttaatcctctatccagacaacacggtgggccaaaggatgaagagaggcatgttggagacctgggcaatgtgactgctggcaaagatggtgtggccaaggtgtctttcgaagattctgtgatctcgctctcaggagaccattccatcattggccgcacattggtggtccatgaaaaagcagatgacttgggcaaaggtggaaatgaagaaagtaaaaagacaggaaacgctggaggtcgtctggcttgtggtgtaattgggatcgcccaataa

SEQ ID NO: 3 - skipped

SEQ ID NO: 4 - DNA, 474 bp, Canis lupus familiaris
  misc_feature (165)..(165): n is a, c, g, or t
cgagtcatggagatgaaggccgtgtgcgtgttgaagggccagggcccggtggagggcaccatccacttcgtgcagaagggaagtgggcctgttgtggtatcaggaaccattacagggctgactgaaggcgagcatggattccacgtccatcagtttgaagataanacacaaggctgtactagtgcaggtcctcactttaatcctctgtccaaaaaacatggtgggccaaaagatcaagagaggcatgttggagacctgggcaatgtgactgctggcaaggatggcgtggccattgtgtccatagaagattctctgattgcactctcaggagactattccatcattggccgcaccatggtggtccacgagaaacgagatgacttgggcaaaggtgacaatgaagaaagtacacagacaggaaacgccgggagtcgtttggcttgtggtgtcattgggatcgcccaataaacattc

SEQ ID NO: 5 - RNA, 21 nt, Artificial Sequence
  Description of Artificial Sequence: Synthetic polynucleotide
ucaccacaagccaaacgacuu

SEQ ID NO: 6 - RNA, 21 nt, Artificial Sequence
  Description of Artificial Sequence: Synthetic polynucleotide
ugauuaaagugaggaccuguu

SEQ ID NO: 7 - RNA, 21 nt, Artificial Sequence
  Description of Artificial Sequence: Synthetic polynucleotide
uauuaaagugaggaccugcuu

SEQ ID NO: 8 - RNA, 21 nt, Artificial Sequence
  Description of Artificial Sequence: Synthetic polynucleotide
uacaccacaagccaaacgauu

SEQ ID NO: 9 - RNA, 21 nt, Artificial Sequence
  Description of Artificial Sequence: Synthetic polynucleotide
gauuaaagugaggaccugcuu

SEQ ID NO: 10 - RNA, 22 nt, Artificial Sequence
  Description of Artificial Sequence: Synthetic polynucleotide
ucaccacaagccaaacgacuuu

SEQ ID NO: 11 - RNA, 21 nt, Artificial Sequence
  Description of Artificial Sequence: Synthetic polynucleotide
ugccagcagucacauugccuu

SEQ ID NO: 12 - RNA, 21 nt, Artificial Sequence
  Description of Artificial Sequence: Synthetic polynucleotide
uaacagaugaguuaagggguu

SEQ ID NO: 13 - RNA, 21 nt, Artificial Sequence
  Description of Artificial Sequence: Synthetic polynucleotide
  misc_feature (20)..(21): nn is a deoxythymidine dinucleotide
uauuaaagugaggaccugcnn

SEQ ID NO: 14 - RNA, 21 nt, Artificial Sequence
  Description of Artificial Sequence: Synthetic polynucleotide
  misc_feature (20)..(21): nn is a deoxythymidine dinucleotide
uacaccacaagccaaacgann

SEQ ID NO: 15 - RNA, 21 nt, Artificial Sequence
  Description of Artificial Sequence: Synthetic polynucleotide
  misc_feature (20)..(21): nn is a deoxythymidine dinucleotide
uuguuuauugggcgaucccnn

SEQ ID NO: 16 - RNA, 21 nt, Artificial Sequence
  Description of Artificial Sequence: Synthetic polynucleotide
  misc_feature (20)..(21): nn is a deoxythymidine dinucleotide
uguuuauugggcgaucccann

SEQ ID NO: 17 - RNA, 21 nt, Artificial Sequence
  Description of Artificial Sequence: Synthetic polynucleotide
  misc_feature (20)..(21): nn is a deoxythymidine dinucleotide
ucaccacaagccaaacgacnn

SEQ ID NO: 18 - RNA, 21 nt, Artificial Sequence
  Description of Artificial Sequence: Synthetic polynucleotide
  misc_feature (20)..(21): nn is a deoxythymidine dinucleotide
ugauuaaagugaggaccugnn

SEQ ID NO: 19 - RNA, 21 nt, Artificial Sequence
  Description of Artificial Sequence: Synthetic polynucleotide
  misc_feature (20)..(21): nn is a deoxythymidine dinucleotide
uuuuauugggcgaucccaann

SEQ ID NO: 20 - RNA, 21 nt, Artificial Sequence
  Description of Artificial Sequence: Synthetic polynucleotide
  misc_feature (20)..(21): nn is a deoxythymidine dinucleotide
ugucagcagucacauugccnn

SEQ ID NO: 21 - RNA, 21 nt, Artificial Sequence
  Description of Artificial Sequence: Synthetic polynucleotide
  misc_feature (20)..(21): nn is a deoxythymidine dinucleotide
ugcgaucccaauuacaccann

SEQ ID NO: 22 - RNA, 21 nt, Artificial Sequence
  Description of Artificial Sequence: Synthetic polynucleotide
gucguuuggcuugugguggcu

SEQ ID NO: 23 - RNA, 21 nt, Artificial Sequence
  Description of Artificial Sequence: Synthetic polynucleotide
cagguccucacuuuaaucgcu

SEQ ID NO: 24 - RNA, 21 nt, Artificial Sequence
  Description of Artificial Sequence: Synthetic polynucleotide
gcagguccucacuuuaaugcc

SEQ ID NO: 25 - RNA, 21 nt, Artificial Sequence
  Description of Artificial Sequence: Synthetic polynucleotide
gcagguccucacuuuaaugcu

SEQ ID NO: 26 - RNA, 21 nt, Artificial Sequence
  Description of Artificial Sequence: Synthetic polynucleotide
ucguuuggcuuguggugugcu

SEQ ID NO: 27 - RNA, 21 nt, Artificial Sequence
  Description of Artificial Sequence: Synthetic polynucleotide
gcagguccucacuuuaauccc

SEQ ID NO: 28 - RNA, 21 nt, Artificial Sequence
  Description of Artificial Sequence: Synthetic polynucleotide
gucguuuggcuugugguggcc

SEQ ID NO: 29 - RNA, 21 nt, Artificial Sequence
  Description of Artificial Sequence: Synthetic polynucleotide
cagguccucacuuuaaucgcc

SEQ ID NO: 30 - RNA, 21 nt, Artificial Sequence
  Description of Artificial Sequence: Synthetic polynucleotide
ucguuuggcuuguggugugcc

SEQ ID NO: 31 - RNA, 21 nt, Artificial Sequence
  Description of Artificial Sequence: Synthetic polynucleotide
ggcaaugugacugcuggugcc

SEQ ID NO: 32 - RNA, 21 nt, Artificial Sequence
  Description of Artificial Sequence: Synthetic polynucleotide
ggcaaugugacugcugguacc

SEQ ID NO: 33 - RNA, 21 nt, Artificial Sequence
  Description of Artificial Sequence: Synthetic polynucleotide
ggcaaugugucugcugguacc

SEQ ID NO: 34 - RNA, 21 nt, Artificial Sequence
  Description of Artificial Sequence: Synthetic polynucleotide
ggcaaugugacugcuggcccc

SEQ ID NO: 35 - RNA, 21 nt, Artificial Sequence
  Description of Artificial Sequence: Synthetic polynucleotide
gcagguccucacuuuaauucc

SEQ ID NO: 36 - RNA, 21 nt, Artificial Sequence
  Description of Artificial Sequence: Synthetic polynucleotide
gcagguccugacuuuaauccc

SEQ ID NO: 37 - RNA, 21 nt, Artificial Sequence
  Description of Artificial Sequence: Synthetic polynucleotide
ccccuuaacucauuuguuccc

SEQ ID NO: 38 - RNA, 21 nt, Artificial Sequence
  Description of Artificial Sequence: Synthetic polynucleotide
  misc_feature (20)..(21): nn is a deoxythymidine dinucleotide
gcagguccucacuuuaaucnn

SEQ ID NO: 39 - RNA, 21 nt, Artificial Sequence
  Description of Artificial Sequence: Synthetic polynucleotide
  misc_feature (20)..(21): nn is a deoxythymidine dinucleotide
ucguuuggcuuguggugucnn

SEQ ID NO: 40 - RNA, 21 nt, Artificial Sequence
  Description of Artificial Sequence: Synthetic polynucleotide
  misc_feature (20)..(21): nn is a deoxythymidine dinucleotide
gggaucgcccaauaaacacnn

SEQ ID NO: 41 - RNA, 21 nt, Artificial Sequence
  Description of Artificial Sequence: Synthetic polynucleotide
  misc_feature (20)..(21): nn is a deoxythymidine dinucleotide
ugggaucgcccaauaaaccnn

SEQ ID NO: 42 - RNA, 21 nt, Artificial Sequence
  Description of Artificial Sequence: Synthetic polynucleotide
  misc_feature (20)..(21): nn is a deoxythymidine dinucleotide
gucguuuggcuuguggugcnn

SEQ ID NO: 43 - RNA, 21 nt, Artificial Sequence
  Description of Artificial Sequence: Synthetic polynucleotide
  misc_feature (20)..(21): nn is a deoxythymidine dinucleotide
cagguccucacuuuaauccnn

SEQ ID NO: 44 - RNA, 21 nt, Artificial Sequence
  Description of Artificial Sequence: Synthetic polynucleotide
  misc_feature (20)..(21): nn is a deoxythymidine dinucleotide
uugggaucgcccaauaaacnn

SEQ ID NO: 45 - RNA, 21 nt, Artificial Sequence
  Description of Artificial Sequence: Synthetic polynucleotide
  misc_feature (20)..(21): nn is a deoxythymidine dinucleotide
ggcaaugugacugcugaccnn

SEQ ID NO: 46 - RNA, 21 nt, Artificial Sequence
  Description of Artificial Sequence: Synthetic polynucleotide
  misc_feature (20)..(21): nn is a deoxythymidine dinucleotide
ugguguaauugggaucgccnn

SEQ ID NO: 47 - DNA, 30 bp, Artificial Sequence
  Description of Artificial Sequence: Synthetic polynucleotide
ctcccgcagaacaccatgcgctccacggaa

SEQ ID NO: 48 - DNA, 100 bp, Artificial Sequence
  Description of Artificial Sequence: Synthetic polynucleotide
gaagcaaagaaggggcagagggagcccgtgagctgagtgggccagggactgggagaaggagtgaggaggcagggccggcatgcctctgctgctggccaga

SEQ ID NO: 49 - DNA, 54 bp, Artificial Sequence
  Description of Artificial Sequence: Synthetic polynucleotide
gtgctgggcggggggcggcgggccctcccgcagaacaccatgcgctcttcggaa

SEQ ID NO: 50 - DNA, 15 bp, Artificial Sequence
  Description of Artificial Sequence: Synthetic polynucleotide
gtggccactgagaag

SEQ ID NO: 51 - DNA, 18 bp, Artificial Sequence
  Description of Artificial Sequence: Synthetic polynucleotide
gtctgcacctgtcactag

SEQ ID NO: 52 - DNA, 10 bp, Artificial Sequence
  Description of Artificial Sequence: Synthetic polynucleotide
tgtgacctgg

SEQ ID NO: 53 - DNA, 10 bp, Artificial Sequence
  Description of Artificial Sequence: Synthetic polynucleotide
tgtgatttgg

SEQ ID NO: 54 - DNA, 35 bp, Artificial Sequence
  Description of Artificial Sequence: Synthetic polynucleotide
ctgaggagcgccttgacagcagccatgggagggcc

SEQ ID NO: 55 - DNA, 100 bp, Artificial Sequence
  Description of Artificial Sequence: Synthetic polynucleotide
tggccgtgtagtgctacccagcgctggctgcctcctcagcattgcaattcctctcccatctgggcaccagtcagctaccctggtgggaatctgggtagcc

SEQ ID NO: 56 - DNA, 99 bp, Artificial Sequence
  Description of Artificial Sequence: Synthetic polynucleotide
ggccgtgtagtgctacccagcgctggctgcctcctcagcattgcaattcctctcccatctgggcaccagtcagctaccctggtgggaatctgggtagcc

SEQ ID NO: 57 - DNA, 52 bp, Artificial Sequence
  Description of Artificial Sequence: Synthetic polynucleotide
ctgaggagcgccttgacagcagccatgggagggccgccccctacctcagtga

SEQ ID NO: 58 - DNA, 52 bp, Artificial Sequence
  Description of Artificial Sequence: Synthetic polynucleotide
ctgtggagcgccttgacagcagccatgggagggccgccccctacctcagtga

SEQ ID NO: 59 - DNA, 158 bp, Artificial Sequence
  Description of Artificial Sequence: Synthetic polynucleotide
gtgctgggcggggggcggcgggccctcccgcagaacaccatgcgctcttcggaagcaggtcctcactttaatgcctgtgacctgggattaaagtgaggacctgcttctgaggagcgccttgacagcagccatgggagggccgccccctacctcagtga

SEQ ID NO: 60 - DNA, 158 bp, Artificial Sequence
  Description of Artificial Sequence: Synthetic polynucleotide
gtgctgggcggggggcggcgggccctcccgcagaacaccatgcgctcttcggaaggcaatgtgactgctggcccctgtgacctggtgccagcagtcacattgccttctgaggagcgccttgacagcagccatgggagggccgccccctacctcagtga

SEQ ID NO: 61 - DNA, 158 bp, Artificial Sequence
  Description of Artificial Sequence: Synthetic polynucleotide
gtgctgggcggggggcggcgggccctcccgcagaacaccatgcgctcttcggaagcaggtcctcactttaattcctgtgacctgggattaaagtgaggacctgcttctgaggagcgccttgacagcagccatgggagggccgccccctacctcagtga

SEQ ID NO: 62 - DNA, 122 bp, Artificial Sequence
  Description of Artificial Sequence: Synthetic polynucleotide
ctcccgcagaacaccatgcgctccacggaagcaggtcctcactttaatgctgtggccactgagaagtattaaagtgaggacctgcttctgaggagcgccttgacagcagccatgggagggcc

SEQ ID NO: 63 - DNA, 122 bp, Artificial Sequence
  Description of Artificial Sequence: Synthetic polynucleotide
ctcccgcagaacaccatgcgctccacggaacaggtcctcactttaatcgctgtggccactgagaagtgattaaagtgaggacctgttctgaggagcgccttgacagcagccatgggagggcc

SEQ ID NO: 64 - DNA, 158 bp, Artificial Sequence
  Description of Artificial Sequence: Synthetic polynucleotide
gtgctgggcggggggcggcgggccctcccgcagaacaccatgcgctcttcggaaggcaatgtgactgctggtgcctgtgacctggtgccagcagtcacattgccttctgaggagcgccttgacagcagccatgggagggccgccccctacctcagtga

SEQ ID NO: 65 - DNA, 122 bp, Artificial Sequence
  Description of Artificial Sequence: Synthetic polynucleotide
ctcccgcagaacaccatgcgctccacggaagtcgtttggcttgtggtggctgtggccactgagaagtcaccacaagccaaacgacttctgaggagcgccttgacagcagccatgggagggcc

SEQ ID NO: 66 - DNA, 122 bp, Artificial Sequence
  Description of Artificial Sequence: Synthetic polynucleotide
ctcccgcagaacaccatgcgctccacggaatcgtttggcttgtggtgtgctgtggccactgagaagtacaccacaagccaaacgattctgaggagcgccttgacagcagccatgggagggcc

SEQ ID NO: 67 - DNA, 158 bp, Artificial Sequence
  Description of Artificial Sequence: Synthetic polynucleotide
gtgctgggcggggggcggcgggccctcccgcagaacaccatgcgctcttcggaagcaggtcctcactttaatccctgtgatttgggattaaagtgaggacctgcttctgaggagcgccttgacagcagccatgggagggccgccccctacctcagtga

SEQ ID NO: 68 - DNA, 158 bp, Artificial Sequence
  Description of Artificial Sequence: Synthetic polynucleotide
gtgctgggcggggggcggcgggccctcccgcagaacaccatgcgctcttcggaaggcaatgtgactgctggtacctgtgatttggtgccagcagtcacattgccttctgaggagcgccttgacagcagccatgggagggccgccccctacctcagtga

SEQ ID NO: 69 - DNA, 158 bp, Artificial Sequence
  Description of Artificial Sequence: Synthetic polynucleotide
gtgctgggcggggggcggcgggccctcccgcagaacaccatgcgctcttcggaagcaggtcctgactttaatccctgtgacctgggattaaagtgaggacctgcttctgtggagcgccttgacagcagccatgggagggccgccccctacctcagtga

SEQ ID NO: 70 - DNA, 158 bp, Artificial Sequence
  Description of Artificial Sequence: Synthetic polynucleotide
gtgctgggcggggggcggcgggccctcccgcagaacaccatgcgctcttcggaaggcaatgtgtctgctggtacctgtgacctggtgccagcagtcacattgccttctgtggagcgccttgacagcagccatgggagggccgccccctacctcagtga

SEQ ID NO: 71 - DNA, 158 bp, Artificial Sequence
  Description of Artificial Sequence: Synthetic polynucleotide
gtgctgggcggggggcggcgggccctcccgcagaacaccatgcgctcttcggaagcaggtcctcactttaatccctgtgacctgggattaaagtgaggacctgcttctgtggagcgccttgacagcagccatgggagggccgccccctacctcagtga

SEQ ID NO: 72 - DNA, 158 bp, Artificial Sequence
  Description of Artificial Sequence: Synthetic polynucleotide
gtgctgggcggggggcggcgggccctcccgcagaacaccatgcgctcttcggaaggcaatgtgactgctggtacctgtgacctggtgccagcagtcacattgccttctgtggagcgccttgacagcagccatgggagggccgccccctacctcagtga

SEQ ID NO: 73 - DNA, 260 bp, Artificial Sequence
  Description of Artificial Sequence: Synthetic polynucleotide
gaagcaaagaaggggcagagggagcccgtgagctgagtgggccagggactgggagaaggagtgaggaggcagggccggcatgcctctgctgctggccagagcaggtcctcactttaatcccgtctgcacctgtcactaggattaaagtgaggacctgctttggccgtgtagtgctacccagcgctggctgcctcctcagcattgcaattcctctcccatctgggcaccagtcagctaccctggtgggaatctgggtagcc

SEQ ID NO: 74 - DNA, 260 bp, Artificial Sequence
  Description of Artificial Sequence: Synthetic polynucleotide
gaagcaaagaaggggcagagggagcccgtgagctgagtgggccagggactgggagaaggagtgaggaggcagggccggcatgcctctgctgctggccagagcaggtcctcactttaatgccgtctgcacctgtcactagtattaaagtgaggacctgctttggccgtgtagtgctacccagcgctggctgcctcctcagcattgcaattcctctcccatctgggcaccagtcagctaccctggtgggaatctgggtagcc

SEQ ID NO: 75 - DNA, 260 bp, Artificial Sequence
  Description of Artificial Sequence: Synthetic polynucleotide
gaagcaaagaaggggcagagggagcccgtgagctgagtgggccagggactgggagaaggagtgaggaggcagggccggcatgcctctgctgctggccagacaggtcctcactttaatcgccgtctgcacctgtcactagtgattaaagtgaggacctgtttggccgtgtagtgctacccagcgctggctgcctcctcagcattgcaattcctctcccatctgggcaccagtcagctaccctggtgggaatctgggtagcc

SEQ ID NO: 76 - DNA, 260 bp, Artificial Sequence
  Description of Artificial Sequence: Synthetic polynucleotide
gaagcaaagaaggggcagagggagcccgtgagctgagtgggccagggactgggagaaggagtgaggaggcagggccggcatgcctctgctgctggccagaggcaatgtgactgctggtaccgtctgcacctgtcactagtgccagcagtcacattgcctttggccgtgtagtgctacccagcgctggctgcctcctcagcattgcaattcctctcccatctgggcaccagtcagctaccctggtgggaatctgggtagcc

SEQ ID NO: 77 - DNA, 260 bp, Artificial Sequence
  Description of Artificial Sequence: Synthetic polynucleotide
gaagcaaagaaggggcagagggagcccgtgagctgagtgggccagggactgggagaaggagtgaggaggcagggccggcatgcctctgctgctggccagagtcgtttggcttgtggtggccgtctgcacctgtcactagtcaccacaagccaaacgactttggccgtgtagtgctacccagcgctggctgcctcctcagcattgcaattcctctcccatctgggcaccagtcagctaccctggtgggaatctgggtagcc

SEQ ID NO: 78 - DNA, 260 bp, Artificial Sequence
  Description of Artificial Sequence: Synthetic polynucleotide
gaagcaaagaaggggcagagggagcccgtgagctgagtgggccagggactgggagaaggagtgaggaggcagggccggcatgcctctgctgctggccagatcgtttggcttgtggtgtgccgtctgcacctgtcactagtacaccacaagccaaacgatttggccgtgtagtgctacccagcgctggctgcctcctcagcattgcaattcctctcccatctgggcaccagtcagctaccctggtgggaatctgggtagcc

SEQ ID NO: 79 - DNA, 260 bp, Artificial Sequence
  Description of Artificial Sequence: Synthetic polynucleotide
gaagcaaagaaggggcagagggagcccgtgagctgagtgggccagggactgggagaaggagtgaggaggcagggccggcatgcctctgctgctggccagaccccttaactcatttgttcccgtctgcacctgtcactagtaacagatgagttaaggggtttggccgtgtagtgctacccagcgctggctgcctcctcagcattgcaattcctctcccatctgggcaccagtcagctaccctggtgggaatctgggtagcc

SEQ ID NO: 80 - DNA, 21 bp, Artificial Sequence
  Description of Artificial Sequence: Synthetic polynucleotide
gcaggtcctcactttaatgcc

SEQ ID NO: 81 - DNA, 21 bp, Artificial Sequence
  Description of Artificial Sequence: Synthetic polynucleotide
ggcaatgtgactgctggcccc

SEQ ID NO: 82 - DNA, 21 bp, Artificial Sequence
  Description of Artificial Sequence: Synthetic polynucleotide
gcaggtcctcactttaattcc

SEQ ID NO: 83 - DNA, 21 bp, Artificial Sequence
  Description of Artificial Sequence: Synthetic polynucleotide
gcaggtcctcactttaatgct

SEQ ID NO: 84 - DNA, 21 bp, Artificial Sequence
  Description of Artificial Sequence: Synthetic polynucleotide
caggtcctcactttaatcgct

SEQ ID NO: 85 - DNA, 21 bp, Artificial Sequence
  Description of Artificial Sequence: Synthetic polynucleotide
ggcaatgtgactgctggtgcc

SEQ ID NO: 86 - DNA, 21 bp, Artificial Sequence
  Description of Artificial Sequence: Synthetic polynucleotide
gtcgtttggcttgtggtggct

SEQ ID NO: 87 - DNA, 21 bp, Artificial Sequence
  Description of Artificial Sequence: Synthetic polynucleotide
tcgtttggcttgtggtgtgct

SEQ ID NO: 88 - DNA, 21 bp, Artificial Sequence
  Description of Artificial Sequence: Synthetic polynucleotide
gcaggtcctcactttaatccc

SEQ ID NO: 89 - DNA, 21 bp, Artificial Sequence
  Description of Artificial Sequence: Synthetic polynucleotide
ggcaatgtgactgctggtacc

SEQ ID NO: 90 - DNA, 21 bp, Artificial Sequence
  Description of Artificial Sequence: Synthetic polynucleotide
gcaggtcctgactttaatccc

SEQ ID NO: 91 - DNA, 21 bp, Artificial Sequence
  Description of Artificial Sequence: Synthetic polynucleotide
ggcaatgtgtctgctggtacc

SEQ ID NO: 92 - DNA, 21 bp, Artificial Sequence
  Description of Artificial Sequence: Synthetic polynucleotide
gcaggtcctcactttaatccc

SEQ ID NO: 93 - DNA, 21 bp, Artificial Sequence
  Description of Artificial Sequence: Synthetic polynucleotide
ggcaatgtgactgctggtacc

SEQ ID NO: 94 - DNA, 21 bp, Artificial Sequence
  Description of Artificial Sequence: Synthetic polynucleotide
gcaggtcctcactttaatccc

SEQ ID NO: 95 - DNA, 21 bp, Artificial Sequence
  Description of Artificial Sequence: Synthetic polynucleotide
gcaggtcctcactttaatgcc

SEQ ID NO: 96 - DNA, 21 bp, Artificial Sequence
  Description of Artificial Sequence: Synthetic polynucleotide
caggtcctcactttaatcgcc

SEQ ID NO: 97 - DNA, 21 bp, Artificial Sequence
  Description of Artificial Sequence: Synthetic polynucleotide
ggcaatgtgactgctggtacc

SEQ ID NO: 98 - DNA, 21 bp, Artificial Sequence
  Description of Artificial Sequence: Synthetic polynucleotide
gtcgtttggcttgtggtggcc

SEQ ID NO: 99 - DNA, 21 bp, Artificial Sequence
  Description of Artificial Sequence: Synthetic polynucleotide
tcgtttggcttgtggtgtgcc

SEQ ID NO: 100 - DNA, 21 bp, Artificial Sequence
  Description of Artificial Sequence: Synthetic polynucleotide
ccccttaactcatttgttccc

SEQ ID NO: 101 - DNA, 21 bp, Artificial Sequence
  Description of Artificial Sequence: Synthetic polynucleotide
gattaaagtgaggacctgctt

SEQ ID NO: 102 - DNA, 21 bp, Artificial Sequence
  Description of Artificial Sequence: Synthetic polynucleotide
tgccagcagtcacattgcctt

SEQ ID NO: 103 - DNA, 21 bp, Artificial Sequence
  Description of Artificial Sequence: Synthetic polynucleotide
gattaaagtgaggacctgctt

SEQ ID NO: 104 - DNA, 21 bp, Artificial Sequence
  Description of Artificial Sequence: Synthetic polynucleotide
tattaaagtgaggacctgctt

SEQ ID NO: 105 - DNA, 21 bp, Artificial Sequence
  Description of Artificial Sequence: Synthetic polynucleotide
tgattaaagtgaggacctgtt

SEQ ID NO: 106 - DNA, 21 bp, Artificial Sequence
  Description of Artificial Sequence: Synthetic polynucleotide
tgccagcagtcacattgcctt

SEQ ID NO: 107 - DNA, 21 bp, Artificial Sequence
  Description of Artificial Sequence: Synthetic polynucleotide
tcaccacaagccaaacgactt

SEQ ID NO: 108 - DNA, 21 bp, Artificial Sequence
  Description of Artificial Sequence: Synthetic polynucleotide
tacaccacaagccaaacgatt

SEQ ID NO: 109 - DNA, 21 bp, Artificial Sequence
  Description of Artificial Sequence: Synthetic polynucleotide
gattaaagtgaggacctgctt

SEQ ID NO: 110 - DNA, 21 bp, Artificial Sequence
  Description of Artificial Sequence: Synthetic polynucleotide
tgccagcagtcacattgcctt

SEQ ID NO: 111 - DNA, 21 bp, Artificial Sequence
  Description of Artificial Sequence: Synthetic polynucleotide
gattaaagtgaggacctgctt

SEQ ID NO: 112 - DNA, 21 bp, Artificial Sequence
  Description of Artificial Sequence: Synthetic polynucleotide
tgccagcagtcacattgcctt

SEQ ID NO: 113 - DNA, 21 bp, Artificial Sequence
  Description of Artificial Sequence: Synthetic polynucleotide
gattaaagtgaggacctgctt

SEQ ID NO: 114 - DNA, 21 bp, Artificial Sequence
  Description of Artificial Sequence: Synthetic polynucleotide
tgccagcagtcacattgcctt

SEQ ID NO: 115 - DNA, 21 bp, Artificial Sequence
  Description of Artificial Sequence: Synthetic polynucleotide
gattaaagtgaggacctgctt

SEQ ID NO: 116 - DNA, 21 bp, Artificial Sequence
  Description of Artificial Sequence: Synthetic polynucleotide
tattaaagtgaggacctgctt

SEQ ID NO: 117 - DNA, 21 bp, Artificial Sequence
  Description of Artificial Sequence: Synthetic polynucleotide
tgattaaagtgaggacctgtt

SEQ ID NO: 118 - DNA, 21 bp, Artificial Sequence
  Description of Artificial Sequence: Synthetic polynucleotide
tgccagcagtcacattgcctt

SEQ ID NO: 119 - DNA, 22 bp, Artificial Sequence
  Description of Artificial Sequence: Synthetic polynucleotide
tcaccacaagccaaacgacttt

SEQ ID NO: 120 - DNA, 21 bp, Artificial Sequence
  Description of Artificial Sequence: Synthetic polynucleotide
tacaccacaagccaaacgatt

SEQ ID NO: 121 - DNA, 21 bp, Artificial Sequence
  Description of Artificial Sequence: Synthetic polynucleotide
taacagatgagttaaggggtt

SEQ ID NO: 122 - DNA, 1453 bp, Artificial Sequence
  Description of Artificial Sequence: Synthetic polynucleotide
ctgcgcgctcgctcgctcactgaggccgcccgggcaaagcccgggcgtcgggcgacctttggtcgcccggcctcagtgagcgagcgagcgcgcagagagggagtgtagccatgctctaggaagatcaattcaattcacgcgtcgacattgattattgactagttattaatagtaatcaattacggggtcattagttcatagcccatatatggagttccgcgttacataacttacggtaaatggcccgcctggctgaccgcccaacgacccccgcccattgacgtcaataatgacgtatgttcccatagtaacgccaatagggactttccattgacgtcaatgggtggagtatttacggtaaactgcccacttggcagtacatcaagtgtatcatatgccaagtacgccccctattgacgtcaatgacggtaaatggcccgcctggcattatgcccagtacatgaccttatgggactttcctacttggcagtacatctacgtattagtcatcgctattaccatgtcgaggccacgttctgcttcactctccccatctcccccccctccccacccccaattttgtatttatttattttttaattattttgtgcagcgatgggggcggggggggggggcgcgcgccaggcggggcggggcggggcgaggggcggggcggggcgaggcggagaggtgcggcggcagccaatcagagcggcgcgctccgaaagtttccttttatggcgaggcggcggcggcggcggccctataaaaagcgaagcgcgcggcgggcgggagcaagcttgaactgaaaaaccagaaagttaactggtaagtttagtctttttgtcttttatttcaggtcccggatccggtggtggtgcaaatcaaagaactgctcctcagtggatgttgcctttacttctaggcctgtacggaagtgttacttctgctctaaaagctgcggaattgtacccgcggccgatccaccggtaccgagctctcccgcagaacaccatgcgctccacggaagtcgtttggcttgtggtggctgtggccactgagaagtcaccacaagccaaacgacttctgaggagcgccttgacagcagccatgggagggcctcgaggacggggtgaactacgcctgaggatccgatctttttccctctgccaaaaattatggggacatcatgaagccccttgagcatctgacttctggctaataaaggaaatttattttcattgcaatagtgtgttggaattttttgtgtctctcactcggcctaggtagataagtagcatggcgggttaatcattaactacaaggaacccctagtgatggagttggccactccctctctgcgcgctcgctcgctcactgaggccgggcgaccaaaggtcgcccgacgcccgggctttgcccgggcggcctcagtgagcgagcgagcgcgcag

SEQ ID NO: 123 - DNA, 1453 bp, Artificial Sequence
  Description of Artificial Sequence: Synthetic polynucleotide
ctgcgcgctcgctcgctcactgaggccgcccgggcaaagcccgggcgtcgggcgacctttggtcgcccggcctcagtgagcgagcgagcgcgcagagagggagtgtagccatgctctaggaagatcaattcaattcacgcgtcgacattgattattgactagttattaatagtaatcaattacggggtcattagttcatagcccatatatggagttccgcgttacataacttacggtaaatggcccgcctggctgaccgcccaacgacccccgcccattgacgtcaataatgacgtatgttcccatagtaacgccaatagggactttccattgacgtcaatgggtggagtatttacggtaaactgcccacttggcagtacatcaagtgtatcatatgccaagtacgccccctattgacgtcaatgacggtaaatggcccgcctggcattatgcccagtacatgaccttatgggactttcctacttggcagtacatctacgtattagtcatcgctattaccatgtcgaggccacgttctgcttcactctccccatctcccccccctccccacccccaattttgtatttatttattttttaattattttgtgcagcgatgggggcggggggggggggcgcgcgccaggcggggcggggcggggcgaggggcggggcggggcgaggcggagaggtgcggcggcagccaatcagagcggcgcgctccgaaagtttccttttatggcgaggcggcggcggcggcggccctataaaaagcgaagcgcgcggcgggcgggagcaagcttgaactgaaaaaccagaaagttaactggtaagtttagtctttttgtcttttatttcaggtcccggatccggtggtggtgcaaatcaaagaactgctcctcagtggatgttgcctttacttctaggcctgtacggaagtgttacttctgctctaaaagctgcggaattgtacccgcggccgatccaccggtaccgagctctcccgcagaacaccatgcgctccacggaacaggtcctcactttaatcgctgtggccactgagaagtgattaaagtgaggacctgttctgaggagcgccttgacagcagccatgggagggcctcgaggacggggtgaactacgcctgaggatccgatctttttccctctgccaaaaattatggggacatcatgaagccccttgagcatctgacttctggctaataaaggaaatttattttcattgcaatagtgtgttggaattttttgtgtctctcactcggcctaggtagataagtagcatggcgggttaatcattaactacaaggaacccctagtgatggagttggccactccctctctgcgcgctcgctcgctcactgaggccgggcgaccaaaggtcgcccgacgcccgggctttgcccgggcggcctcagtgagcgagcgagcgcgcag

SEQ ID NO: 124 - DNA, 1584 bp, Artificial Sequence
  Description of Artificial Sequence: Synthetic polynucleotide
ctgcgcgctcgctcgctcactgaggccgcccgggcaaagcccgggcgtcgggcgacctttggtcgcccggcctcagtgagcgagcgagcgcgcagagagggagtgtagccatgctctaggaagatcaattcaattcacgcgtcgacattgattattgactagttattaatagtaatcaattacggggtcattagttcatagcccatatatggagttccgcgttacataacttacggtaaatggcccgcctggctgaccgcccaacgacccccgcccattgacgtcaataatgacgtatgttcccatagtaacgccaatagggactttccattgacgtcaatgggtggagtatttacggtaaactgcccacttggcagtacatcaagtgtatcatatgccaagtacgccccctattgacgtcaatgacggtaaatggcccgcctggcattatgcccagtacatgaccttatgggactttcctacttggcagtacatctacgtattagtcatcgctattaccatgtcgaggccacgttctgcttcactctccccatctcccccccctccccacccccaattttgtatttatttattttttaattattttgtgcagcgatgggggcggggggggggggcgcgcgccaggcggggcggggcggggcgaggggcggggcggggcgaggcggagaggtgcggcggcagccaatcagagcggcgcgctccgaaagtttccttttatggcgaggcggcggcggcggcggccctataaaaagcgaagcgcgcggcgggcgggagcaagcttgaactgaaaaaccagaaagttaactggtaagtttagtctttttgtcttttatttcaggtcccggatccggtggtggtgcaaatcaaagaactgctcctcagtggatgttgcctttacttctaggcctgtacggaagtgttacttctgctctaaaagctgcggaattgtacccgcggccgatccaccggtgaagcaaagaaggggcagagggagcccgtgagctgagtgggccagggactgggagaaggagtgaggaggcagggccggcatgcctctgctgctggccagagcaggtcctcactttaatgccgtctgcacctgtcactagtattaaagtgaggacctgctttggccgtgtagtgctacccagcgctggctgcctcctcagcattgcaattcctctcccatctgggcaccagtcagctaccctggtgggaatctgggtagccctcgaggacggggtgaactacgcctgaggatccgatctttttccctctgccaaaaattatggggacatcatgaagccccttgagcatctgacttctggctaataaaggaaatttattttcattgcaatagtgtgttggaattttttgtgtctctcactcggcctaggtagataagtagcatggcgggttaatcattaactacaaggaacccctagtgatggagttggccactccctctctgcgcgctcgctcgctcactgaggccgggcgaccaaaggtcgcccgacgcccgggctttgcccgggcggcctcagtgagcgagcgagcgcgcag

SEQ ID NO: 125 - DNA, 1453 bp, Artificial Sequence
  Description of Artificial Sequence: Synthetic polynucleotide
ctgcgcgctcgctcgctcactgaggccgcccgggcaaagcccgggcgtcgggcgacctttggtcgcccggcctcagtgagcgagcgagcgcgcagagagggagtgtagccatgctctaggaagatcaattcaattcacgcgtcgacattgattattgactagttattaatagtaatcaattacggggtcattagttcatagcccatatatggagttccgcgttacataacttacggtaaatggcccgcctggctgaccgcccaacgacccccgcccattgacgtcaataatgacgtatgttcccatagtaacgccaatagggactttccattgacgtcaatgggtggagtatttacggtaaactgcccacttggcagtacatcaagtgtatcatatgccaagtacgccccctattgacgtcaatgacggtaaatggcccgcctggcattatgcccagtacatgaccttatgggactttcctacttggcagtacatctacgtattagtcatcgctattaccatgtcgaggccacgttctgcttcactctccccatctcccccccctccccacccccaattttgtatttatttattttttaattattttgtgcagcgatgggggcggggggggggggcgcgcgccaggcggggcggggcggggcgaggggcggggcggggcgaggcggagaggtgcggcggcagccaatcagagcggcgcgctccgaaagtttccttttatggcgaggcggcggcggcggcggccctataaaaagcgaagcgcgcggcgggcgggagcaagcttgaactgaaaaaccagaaagttaactggtaagtttagtctttttgtcttttatttcaggtcccggatccggtggtggtgcaaatcaaagaactgctcctcagtggatgttgcctttacttctaggcctgtacggaagtgttacttctgctctaaaagctgcggaattgtacccgcggccgatccaccggtaccgagctctcccgcagaacaccatgcgctccacggaagcaggtcctcactttaatgctgtggccactgagaagtattaaagtgaggacctgcttctgaggagcgccttgacagcagccatgggagggcctcgaggacggggtgaactacgcctgaggatccgatctttttccctctgccaaaaattatggggacatcatgaagccccttgagcatctgacttctggctaataaaggaaatttattttcattgcaatagtgtgttggaattttttgtgtctctcactcggcctaggtagataagtagcatggcgggttaatcattaactacaaggaacccctagtgatggagttggccactccctctctgcgcgctcgctcgctcactgaggccgggcgaccaaaggtcgcccgacgcccgggctttgcccgggcggcctcagtgagcgagcgagcgcgcag

SEQ ID NO: 126 - DNA, 1453 bp, Artificial Sequence
  Description of Artificial Sequence: Synthetic polynucleotide
ctgcgcgctcgctcgctcactgaggccgcccgggcaaagcccgggcgtcgggcgacctttggtcgcccggcctcagtgagcgagcgagcgcgcagagagggagtgtagccatgctctaggaagatcaattcaattcacgcgtcgacattgattattgactagttattaatagtaatcaattacggggtcattagttcatagcccatatatggagttccgcgttacataacttacggtaaatggcccgcctggctgaccgcccaacgacccccgcccattgacgtcaataatgacgtatgttcccatagtaacgccaatagggactttccattgacgtcaatgggtggagtatttacggtaaactgcccacttggcagtacatcaagtgtatcatatgccaagtacgccccctattgacgtcaatgacggtaaatggcccgcctggcattatgcccagtacatgaccttatgggactttcctacttggcagtacatctacgtattagtcatcgctattaccatgtcgaggccacgttctgcttcactctccccatctcccccccctccccacccccaattttgtatttatttattttttaattattttgtgcagcgatgggggcggggggggggggcgcgcgccaggcggggcggggcggggcgaggggcggggcggggcgaggcggagaggtgcggcggcagccaatcagagcggcgcgctccgaaagtttccttttatggcgaggcggcggcggcggcggccctataaaaagcgaagcgcgcggcgggcgggagcaagcttgaactgaaaaaccagaaagttaactggtaagtttagtctttttgtcttttatttcaggtcccggatccggtggtggtgcaaatcaaagaactgctcctcagtggatgttgcctttacttctaggcctgtacggaagtgttacttctgctctaaaagctgcggaattgtacccgcggccgatccaccggtaccgagctctcccgcagaacaccatgcgctccacggaatcgtttggcttgtggtgtgctgtggccactgagaagtacaccacaagccaaacgattctgaggagcgccttgacagcagccatgggagggcctcgaggacggggtgaactacgcctgaggatccgatctttttccctctgccaaaaattatggggacatcatgaagccccttgagcatctgacttctggctaataaaggaaatttattttcattgcaatagtgtgttggaattttttgtgtctctcactcggcctaggtagataagtagcatggcgggttaatcattaactacaaggaacccctagtgatggagttggccactccctctctgcgcgctcgctcgctcactgaggccgggcgaccaaaggtcgcccgacgcccgggctttgcccgggcggcctcagtgagcgagcgagcgcgcag

SEQ ID NO: 127 - DNA, 1584 bp, Artificial Sequence
  Description of Artificial Sequence: Synthetic polynucleotide
ctgcgcgctcgctcgctcactgaggccgcccgggcaaagcccgggcgtcgggcgacctttggtcgcccggcctcagtgagcgagcgagcgcgcagagagggagtgtagccatgctctaggaagatcaattcaattcacgcgtcgacattgattattgactagttattaatagtaatcaattacggggtcattagttcatagcccatatatggagttccgcgttacataacttacggtaaatggcccgcctggctgaccgcccaacgacccccgcccattgacgtcaataatgacgtatgttcccatagtaacgccaatagggactttccattgacgtcaatgggtggagtatttacggtaaactgcccacttggcagtacatcaagtgtatcatatgccaagtacgccccctattgacgtcaatgacggtaaatggcccgcctggcattatgcccagtacatgaccttatgggactttcctacttggcagtacatctacgtattagtcatcgctattaccatgtcgaggccacgttctgcttcactctccccatctcccccccctccccacccccaattttgtatttatttattttttaattattttgtgcagcgatgggggcggggggggggggcgcgcgccaggcggggcggggcggggcgaggggcggggcggggcgaggcggagaggtgcggcggcagccaatcagagcggcgcgctccgaaagtttccttttatggcgaggcggcggcggcggcggccctataaaaagcgaagcgcgcggcgggcgggagcaagcttgaactgaaaaaccagaaagttaactggtaagtttagtctttttgtcttttatttcaggtcccggatccggtggtggtgcaaatcaaagaactgctcctcagtggatgttgcctttacttctaggcctgtacggaagtgttacttctgctctaaaagctgcggaattgtacccgcggccgatccaccggtgaagcaaagaaggggcagagggagcccgtgagctgagtgggccagggactgggagaaggagtgaggaggcagggccggcatgcctctgctgctggccagagcaggtcctcactttaatcccgtctgcacctgtcactaggattaaagtgaggacctgctttggccgtgtagtgctacccagcgctggctgcctcctcagcattgcaattcctctcccatctgggcaccagtcagctaccctggtgggaatctgggtagccctcgaggacggggtgaactacgcctgaggatccgatctttttccctctgccaaaaattatggggacatcatgaagccccttgagcatctgacttctggctaataaaggaaatttattttcattgcaatagtgtgttggaattttttgtgtctctcactcggcctaggtagataagtagcatggcgggttaatcattaactacaaggaacccctagtgatggagttggccactccctctctgcgcgctcgctcgctcactgaggccgggcgaccaaaggtcgcccgacgcccgggctttgcccgggcggcctcagtgagcgagcgagcgcgcag

SEQ ID NO: 128 - DNA, 1406 bp, Artificial Sequence
  Description of Artificial Sequence: Synthetic polynucleotide
ctgcgcgctcgctcgctcactgaggccgcccgggcaaagcccgggcgtcgggcgacctttggtcgcccggcctcagtgagcgagcgagcgcgcagagagggagtgtagccatgctctaggaagatcaattcaattcacgcgtccatggcttagaaggcaagaatcctggctgtggaaagatacctaaaggatcaacagctcctggggatttggggttgctctggaaaactcatttgcaccactgctgtgccttggaatgctagttggagtaataaatctctggaacagatttggaatcacacgacctggatggagtgggacagagaaattaacaattacacaagcttaatacactccttaattgaagaatcgcaaaaccagcaagaaaagaatgaacaagaattattggaattagataaatgggcaagtttgtggaattggtttaacataacaaattggctgtggtatataaaattattcataatgatagtaggaggcttggtaggtttaagaatagtttttgctgtactttctatagtgaatagagttaggcagggatattcaccattatcgtttcagacccacctcccaaccccgaggggacccgacaggcccgaaggaatagaagaagaaggtggagagagagacagagacagatccattcgattagtgaacggatctcgacggtatcgatcacgagactagcctcgagcggccgcaattcgaacgctgacgtcatcaacccgctccaaggaatcgcgggcccagtgtcactaggcgggaacacccagcgcgcgtgcgccctggcaggaagatggctgtgagggacagggagtggcgccctgcaatatttgcatgtcgctatgtgttctgggaaatcaccataaacgtgaaatgtctttggatttgggaatcttataagttctgtatgagaccacaccggtaccgagctctcccgcagaacaccatgcgctccacggaagcaggtcctcactttaatgctgtggccactgagaagtattaaagtgaggacctgcttctgaggagcgccttgacagcagccatgggagggcctcgaggacggggtgaactacgcctgaggatccgatctttttccctctgccaaaaattatggggacatcatgaagccccttgagcatctgacttctggctaataaaggaaatttattttcattgcaatagtgtgttggaattttttgtgtctctcactcggcctaggtagataagtagcatggcgggttaatcattaactacaaggaacccctagtgatggagttggccactccctctctgcgcgctcgctcgctcactgaggccgggcgaccaaaggtcgcccgacgcccgggctttgcccgggcggcctcagtgagcgagcgagcgcgcag

SEQ ID NO: 129 - DNA, 1406 bp, Artificial Sequence
  Description of Artificial Sequence: Synthetic polynucleotide
ctgcgcgctcgctcgctcactgaggccgcccgggcaaagcccgggcgtcgggcgacctttggtcgcccggcctcagtgagcgagcgagcgcgcagagagggagtgtagccatgctctaggaagatcaattcaattcacgcgtccatggcttagaaggcaagaatcctggctgtggaaagatacctaaaggatcaacagctcctggggatttggggttgctctggaaaactcatttgcaccactgctgtgccttggaatgctagttggagtaataaatctctggaacagatttggaatcacacgacctggatggagtgggacagagaaattaacaattacacaagcttaatacactccttaattgaagaatcgcaaaaccagcaagaaaagaatgaacaagaattattggaattagataaatgggcaagtttgtggaattggtttaacataacaaattggctgtggtatataaaattattcataatgatagtaggaggcttggtaggtttaagaatagtttttgctgtactttctatagtgaatagagttaggcagggatattcaccattatcgtttcagacccacctcccaaccccgaggggacccgacaggcccgaaggaatagaagaagaaggtggagagagagacagagacagatccattcgattagtgaacggatctcgacggtatcgatcacgagactagcctcgagcggccgcaattcgaacgctgacgtcatcaacccgctccaaggaatcgcgggcccagtgtcactaggcgggaacacccagcgcgcgtgcgccctggcaggaagatggctgtgagggacagggagtggcgccctgcaatatttgcatgtcgctatgtgttctgggaaatcaccataaacgtgaaatgtctttggatttgggaatcttataagttctgtatgagaccacaccggtaccgagctctcccgcagaacaccatgcgctccacggaagtcgtttggcttgtggtggctgtggccactgagaagtcaccacaagccaaacgacttctgaggagcgccttgacagcagccatgggagggcctcgaggacggggtgaactacgcctgaggatccgatctttttccctctgccaaaaattatggggacatcatgaagccccttgagcatctgacttctggctaataaaggaaatttattttcattgcaatagtgtgttggaattttttgtgtctctcactcggcctaggtagataagtagcatggcgggttaatcattaactacaaggaacccctagtgatggagttggccactccctctctgcgcgctcgctcgctcactgaggccgggcgaccaaaggtcgcccgacgcccgggctttgcccgggcggcctcagtgagcgagcgagcgcgcag

SEQ ID NO: 130 - DNA, 1584 bp, Artificial Sequence
  Description of Artificial Sequence: Synthetic polynucleotide
ctgcgcgctcgctcgctcactgaggccgcccgggcaaagcccgggcgtcgggcgacctttggtcgcccggcctcagtgagcgagcgagcgcgcagagagggagtgtagccatgctctaggaagatcaattcaattcacgcgtcgacattgattattgactagttattaatagtaatcaattacggggtcattagttcatagcccatatatggagttccgcgttacataacttacggtaaatggcccgcctggctgaccgcccaacgacccccgcccattgacgtcaataatgacgtatgttcccatagtaacgccaatagggactttccattgacgtcaatgggtggagtatttacggtaaactgcccacttggcagtacatcaagtgtatcatatgccaagtacgccccctattgacgtcaatgacggtaaatggcccgcctggcattatgcccagtacatgaccttatgggactttcctacttggcagtacatctacgtattagtcatcgctattaccatgtcgaggccacgttctgcttcactctccccatctcccccccctccccacccccaattttgtatttatttattttttaattattttgtgcagcgatgggggcggggggggggggcgcgcgccaggcggggcggggcggggcgaggggcggggcggggcgaggcggagaggtgcggcggcagccaatcagagcggcgcgctccgaaagtttccttttatggcgaggcggcggcggcggcggccctataaaaagcgaagcgcgcggcgggcgggagcaagcttgaactgaaaaaccagaaagttaactggtaagtttagtctttttgtcttttatttcaggtcccggatccggtggtggtgcaaatcaaagaactgctcctcagtggatgttgcctttacttctaggcctgtacggaagtgttacttctgctctaaaagctgcggaattgtacccgcggccgatccaccggtgaagcaaagaaggggcagagggagcccgtgagctgagtgggccagggactgggagaaggagtgaggaggcagggccggcatgcctctgctgctggccagagtcgtttggcttgtggtggccgtctgcacctgtcactagtcaccacaagccaaacgactttggccgtgtagtgctacccagcgctggctgcctcctcagcattgcaattcctctcccatctgggcaccagtcagctaccctggtgggaatctgggtagccctcgaggacggggtgaactacgcctgaggatccgatctttttccctctgccaaaaattatggggacatcatgaagccccttgagcatctgacttctggctaataaaggaaatttattttcattgcaatagtgtgttggaattttttgtgtctctcactcggcctaggtagataagtagcatggcgggttaatcattaactacaaggaacccctagtgatggagttggccactccctctctgcgcgctcgctcgctcactgaggccgggcgaccaaaggtcgcccgacgcccgggctttgcccgggcggcctcagtgagcgagcgagcgcgcag

SEQ ID NO: 131 - DNA, 1584 bp, Artificial Sequence
  Description of Artificial Sequence: Synthetic polynucleotide
ctgcgcgctcgctcgctcactgaggccgcccgggcaaagcccgggcgtcgggcgacctttggtcgcccggcctcagtgagcgagcgagcgcgcagagagggagtgtagccatgctctaggaagatcaattcaattcacgcgtcgacattgattattgactagttattaatagtaatcaattacggggtcattagttcatagcccatatatggagttccgcgttacataacttacggtaaatggcccgcctggctgaccgcccaacgacccccgcccattgacgtcaataatgacgtatgttcccatagtaacgccaatagggactttccattgacgtcaatgggtggagtatttacggtaaactgcccacttggcagtacatcaagtgtatcatatgccaagtacgccccctattgacgtcaatgacggtaaatggcccgcctggcattatgcccagtacatgaccttatgggactttcctacttggcagtacatctacgtattagtcatcgctattaccatgtcgaggccacgttctgcttcactctccccatctcccccccctccccacccccaattttgtatttatttattttttaattattttgtgcagcgatgggggcggggggggggggcgcgcgccaggcggggcggggcggggcgaggggcggggcggggcgaggcggagaggtgcggcggcagccaatcagagcggcgcgctccgaaagtttccttttatggcgaggcggcggcggcggcggccctataaaaagcgaagcgcgcggcgggcgggagcaagcttgaactgaaaaaccagaaagttaactggtaagtttagtctttttgtcttttatttcaggtcccggatccggtggtggtgcaaatcaaagaactgctcctcagtggatgttgcctttacttctaggcctgtacggaagtgttacttctgctctaaaagctgcggaattgtacccgcggccgatccaccggtgaagcaaagaaggggcagagggagcccgtgagctgagtgggccagggactgggagaaggagtgaggaggcagggccggcatgcctctgctgctggccagacaggtcctcactttaatcgccgtctgcacctgtcactagtgattaaagtgaggacctgtttggccgtgtagtgctacccagcgctggctgcctcctcagcattgcaattcctctcccatctgggcaccagtcagctaccctggtgggaatctgggtagccctcgaggacggggtgaactacgcctgaggatccgatctttttccctctgccaaaaattatggggacatcatgaagccccttgagcatctgacttctggctaataaaggaaatttattttcattgcaatagtgtgttggaattttttgtgtctctcactcggcctaggtagataagtagcatggcgggttaatcattaactacaaggaacccctagtgatggagttggccactccctctctgcgcgctcgctcgctcactgaggccgggcgaccaaaggtcgcccgacgcccgggctttgcccgggcggcctcagtgagcgagcgagcgcgcag

SEQ ID NO: 132 - DNA, 1584 bp, Artificial Sequence
  Description of Artificial Sequence: Synthetic polynucleotide
ctgcgcgctcgctcgctcactgaggccgcccgggcaaagcccgggcgtcgggcgacctttggtcgcccggcctcagtgagcgagcgagcgcgcagagagggagtgtagccatgctctaggaagatcaattcaattcacgcgtcgacattgattattgactagttattaatagtaatcaattacggggtcattagttcatagcccatatatggagttccgcgttacataacttacggtaaatggcccgcctggctgaccgcccaacgacccccgcccattgacgtcaataatgacgtatgttcccatagtaacgccaatagggactttccattgacgtcaatgggtggagtatttacggtaaactgcccacttggcagtacatcaagtgtatcatatgccaagtacgccccctattgacgtcaatgacggtaaatggcccgcctggcattatgcccagtacatgaccttatgggactttcctacttggcagtacatctacgtattagtcatcgctattaccatgtcgaggccacgttctgcttcactctccccatctcccccccctccccacccccaattttgtatttatttattttttaattattttgtgcagcgatgggggcggggggggggggcgcgcgccaggcggggcggggcggggcgaggggcggggcggggcgaggcggagaggtgcggcggcagccaatcagagcggcgcgctccgaaagtttccttttatggcgaggcggcggcggcggcggccctataaaaagcgaagcgcgcggcgggcgggagcaagcttgaactgaaaaaccagaaagttaactggtaagtttagtctttttgtcttttatttcaggtcccggatccggtggtggtgcaaatcaaagaactgctcctcagtggatgttgcctttacttctaggcctgtacggaagtgttacttctgctctaaaagctgcggaattgtacccgcggccgatccaccggtgaagcaaagaaggggcagagggagcccgtgagctgagtgggccagggactgggagaaggagtgaggaggcagggccggcatgcctctgctgctggccagatcgtttggcttgtggtgtgccgtctgcacctgtcactagtacaccacaagccaaacgatttggccgtgtagtgctacccagcgctggctgcctcctcagcattgcaattcctctcccatctgggcaccagtcagctaccctggtgggaatctgggtagccctcgaggacggggtgaactacgcctgaggatccgatctttttccctctgccaaaaattatggggacatcatgaagccccttgagcatctgacttctggctaataaaggaaatttattttcattgcaatagtgtgttggaattttttgtgtctctcactcggcctaggtagataagtagcatggcgggttaatcattaactacaaggaacccctagtgatggagttggccactccctctctgcgcgctcgctcgctcactgaggccgggcgaccaaaggtcgcccgacgcccgggctttgcccgggcggcctcagtgagcgagcgagcgcgcag

SEQ ID NO: 133 - DNA, 1490 bp, Artificial Sequence
  Description of Artificial Sequence: Synthetic polynucleotide
ctgcgcgctcgctcgctcactgaggccgcccgggcaaagcccgggcgtcgggcgacctttggtcgcccggcctcagtgagcgagcgagcgcgcagagagggagtgtagccatgctctaggaagatcaattcaattcacgcgtcgacattgattattgactagttattaatagtaatcaattacggggtcattagttcatagcccatatatggagttccgcgttacataacttacggtaaatggcccgcctggctgaccgcccaacgacccccgcccattgacgtcaataatgacgtatgttcccatagtaacgccaatagggactttccattgacgtcaatgggtggagtatttacggtaaactgcccacttggcagtacatcaagtgtatcatatgccaagtacgccccctattgacgtcaatgacggtaaatggcccgcctggcattatgcccagtacatgaccttatgggactttcctacttggcagtacatctacgtattagtcatcgctattaccatgtcgaggccacgttctgcttcactctccccatctcccccccctccccacccccaattttgtatttatttattttttaattattttgtgcagcgatgggggcggggggggggggcgcgcgccaggcggggcggggcggggcgaggggcggggcggggcgaggcggagaggtgcggcggcagccaatcagagcggcgcgctccgaaagtttccttttatggcgaggcggcggcggcggcggccctataaaaagcgaagcgcgcggcgggcgggagcaagcttgaactgaaaaaccagaaagttaactggtaagtttagtctttttgtcttttatttcaggtcccggatccggtggtggtgcaaatcaaagaactgctcctcagtggatgttgcctttacttctaggcctgtacggaagtgttacttctgctctaaaagctgcggaattgtacccgcggccgatccaccggtaccgagctgtgctgggcggggggcggcgggccctcccgcagaacaccatgcgctcttcggaaggcaatgtgactgctggtgcctgtgacctggtgccagcagtcacattgccttctgaggagcgccttgacagcagccatgggagggccgccccctacctcagtgactcgaggacggggtgaactacgcctgaggatccgatctttttccctctgccaaaaattatggggacatcatgaagccccttgagcatctgacttctggctaataaaggaaatttattttcattgcaatagtgtgttggaattttttgtgtctctcactcggcctaggtagataagtagcatggcgggttaatcattaactacaaggaacccctagtgatggagttggccactccctctctgcgcgctcgctcgctcactgaggccgggcgaccaaaggtcgcccgacgcccgggctttgcccgggcggcctcagtgagcgagcgagcgcgcag

SEQ ID NO: 134 - DNA, 1490 bp, Artificial Sequence
  Description of Artificial Sequence: Synthetic polynucleotide
ctgcgcgctcgctcgctcactgaggccgcccgggcaaagcccgggcgtcgggcgacctttggtcgcccggcctcagtgagcgagcgagcgcgcagagagggagtgtagccatgctctaggaagatcaattcaattcacgcgtcgacattgattattgactagttattaatagtaatcaattacggggtcattagttcatagcccatatatggagttccgcgttacataacttacggtaaatggcccgcctggctgaccgcccaacgacccccgcccattgacgtcaataatgacgtatgttcccatagtaacgccaatagggactttccattgacgtcaatgggtggagtatttacggtaaactgcccacttggcagtacatcaagtgtatcatatgccaagtacgccccctattgacgtcaatgacggtaaatggcccgcctggcattatgcccagtacatgaccttatgggactttcctacttggcagtacatctacgtattagtcatcgctattaccatgtcgaggccacgttctgcttcactctccccatctcccccccctccccacccccaattttgtatttatttattttttaattattttgtgcagcgatgggggcggggggggggggcgcgcgccaggcggggcggggcggggcgaggggcggggcggggcgaggcggagaggtgcggcggcagccaatcagagcggcgcgctccgaaagtttccttttatggcgaggcggcggcggcggcggccctataaaaagcgaagcgcgcggcgggcgggagcaagcttgaactgaaaaaccagaaagttaactggtaagtttagtctttttgtcttttatttcaggtcccggatccggtggtggtgcaaatcaaagaactgctcctcagtggatgttgcctttacttctaggcctgtacggaagtgttacttctgctctaaaagctgcggaattgtacccgcggccgatccaccggtaccgagctgtgctgggcggggggcggcgggccctcccgcagaacaccatgcgctcttcggaaggcaatgtgactgctggtacctgtgatttggtgccagcagtcacattgccttctgaggagcgccttgacagcagccatgggagggccgccccctacctcagtgactcgaggacggggtgaactacgcctgaggatccgatctttttccctctgccaaaaattatggggacatcatgaagccccttgagcatctgacttctggctaataaaggaaatttattttcattgcaatagtgtgttggaattttttgtgtctctcactcggcctaggtagataagtagcatggcgggttaatcattaactacaaggaacccctagtgatggagttggccactccctctctgcgcgctcgctcgctcactgaggccgggcgaccaaaggtcgcccgacgcccgggctttgcccgggcggcctcagtgagcgagcgagcgcgcag

SEQ ID NO: 135 - DNA, 1490 bp, Artificial Sequence
  Description of Artificial Sequence: Synthetic polynucleotide
ctgcgcgctcgctcgctcactgaggccgcccgggcaaagcccgggcgtcgggcgacctttggtcgcccggcctcagtgagcgagcgagcgcgcagagagggagtgtagccatgctctaggaagatcaattcaattcacgcgtcgacattgattattgactagttattaatagtaatcaattacggggtcattagttcatagcccatatatggagttccgcgttacataacttacggtaaatggcccgcctggctgaccgcccaacgacccccgcccattgacgtcaataatgacgtatgttcccatagtaacgccaatagggactttccattgacgtcaatgggtggagtatttacggtaaactgcccacttggcagtacatcaagtgtatcatatgccaagtacgccccctattgacgtcaatgacggtaaatggcccgcctggcattatgcccagtacatgaccttatgggactttcctacttggcagtacatctacgtattagtcatcgctattaccatgtcgaggccacgttctgcttcactctccccatctcccccccctccccacccccaattttgtatttatttattttttaattattttgtgcagcgatgggggcggggggggggggcgcgcgccaggcggggcggggcggggcgaggggcggggcggggcgaggcggagaggtgcggcggcagccaatcagagcggcgcgctccgaaagtttccttttatggcgaggcggcggcggcggcggccctataaaaagcgaagcgcgcggcgggcgggagcaagcttgaactgaaaaaccagaaagttaactggtaagtttagtctttttgtcttttatttcaggtcccggatccggtggtggtgcaaatcaaagaactgctcctcagtggatgttgcctttacttctaggcctgtacggaagtgttacttctgctctaaaagctgcggaattgtacccgcggccgatccaccggtaccgagctgtgctgggcggggggcggcgggccctcccgcagaacaccatgcgctcttcggaaggcaatgtgactgctggtacctgtgacctggtgccagcagtcacattgccttctgtggagcgccttgacagcagccatgggagggccgccccctacctcagtgactcgaggacggggtgaactacgcctgaggatccgatctttttccctctgccaaaaattatggggacatcatgaagccccttgagcatctgacttctggctaataaaggaaatttattttcattgcaatagtgtgttggaattttttgtgtctctcactcggcctaggtagataagtagcatggcgggttaatcattaactacaaggaacccctagtgatggagttggccactccctctctgcgcgctcgctcgctcactgaggccgggcgaccaaaggtcgcccgacgcccgggctttgcccgggcggcctcagtgagcgagcgagcgcgcag

SEQ ID NO: 136 - DNA, 1490 bp, Artificial Sequence
  Description of Artificial Sequence: Synthetic polynucleotide
ctgcgcgctcgctcgctcactgaggccgcccgggcaaagcccgggcgtcgggcgacctttggtcgcccggcctcagtgagcgagcgagcgcgcagagagggagtgtagccatgctctaggaagatcaattcaattcacgcgtcgacattgattattgactagttattaatagtaatcaattacggggtcattagttcatagcccatatatggagttccgcgttacataacttacggtaaatggcccgcctggctgaccgcccaacgacccccgcccattgacgtcaataatgacgtatgttcccatagtaacgccaatagggactttccattgacgtcaatgggtggagtatttacggtaaactgcccacttggcagtacatcaagtgtatcatatgccaagtacgccccctattgacgtcaatgacggtaaatggcccgcctggcattatgcccagtacatgaccttatgggactttcctacttggcagtacatctacgtattagtcatcgctattaccatgtcgaggccacgttctgcttcactctccccatctcccccccctccccacccccaattttgtatttatttattttttaattattttgtgcagcgatgggggcggggggggggggcgcgcgccaggcggggcggggcggggcgaggggcggggcggggcgaggcggagaggtgcggcggcagccaatcagagcggcgcgctccgaaagtttccttttatggcgaggcggcggcggcggcggccctataaaaagcgaagcgcgcggcgggcgggagcaagcttgaactgaaaaaccagaaagttaactggtaagtttagtctttttgtcttttatttcaggtcccggatccggtggtggtgcaaatcaaagaactgctcctcagtggatgttgcctttacttctaggcctgtacggaagtgttacttctgctctaaaagctgcggaattgtacccgcggccgatccaccggtaccgagctgtgctgggcggggggcggcgggccctcccgcagaacaccatgcgctcttcggaaggcaatgtgtctgctggtacctgtgacctggtgccagcagtcacattgccttctgtggagcgccttgacagcagccatgggagggccgccccctacctcagtgactcgaggacggggtgaactacgcctgaggatccgatctttttccctctgccaaaaattatggggacatcatgaagccccttgagcatctgacttctggctaataaaggaaatttattttcattgcaatagtgtgttggaattttttgtgtctctcactcggcctaggtagataagtagcatggcgggttaatcattaactacaaggaacccctagtgatggagttggccactccctctctgcgcgctcgctcgctcactgaggccgggcgaccaaaggtcgcccgacgcccgggctttgcccgggcggcctcagtgagcgagcgagcgcgcag

SEQ ID NO: 137 - DNA, 1490 bp, Artificial Sequence
  Description of Artificial Sequence: Synthetic polynucleotide
ctgcgcgctcgctcgctcactgaggccgcccgggcaaagcccgggcgtcgggcgacctttggtcgcccggcctcagtgagcgagcgagcgcgcagagagggagtgtagccatgctctaggaagatcaattcaattcacgcgtcgacattgattattgactagttattaatagtaatcaattacggggtcattagttcatagcccatatatggagttccgcgttacataacttacggtaaatggcccgcctggctgaccgcccaacgacccccgcccattgacgtcaataatgacgtatgttcccatagtaacgccaatagggactttccattgacgtcaatgggtggagtatttacggtaaactgcccacttggcagtacatcaagtgtatcatatgccaagtacgccccctattgacgtcaatgacggtaaatggcccgcctggcattatgcccagtacatgaccttatgggactttcctacttggcagtacatctacgtattagtcatcgctattaccatgtcgaggccacgttctgcttcactctccccatctcccccccctccccacccccaattttgtatttatttattttttaattattttgtgcagcgatgggggcggggggggggggcgcgcgccaggcggggcggggcggggcgaggggcggggcggggcgaggcggagaggtgcggcggcagccaatcagagcggcgcgctccgaaagtttccttttatggcgaggcggcggcggcggcggccctataaaaagcgaagcgcgcggcgggcgggagcaagcttgaactgaaaaaccagaaagttaactggtaagtttagtctttttgtcttttatttcaggtcccggatccggtggtggtgcaaatcaaagaactgctcctcagtggatgttgcctttacttctaggcctgtacggaagtgttacttctgctctaaaagctgcggaattgtacccgcggccgatccaccggtaccgagctgtgctgggcggggggcggcgggccctcccgcagaacaccatgcgctcttcggaaggcaatgtgactgctggcccctgtgacctggtgccagcagtcacattgccttctgaggagcgccttgacagcagccatgggagggccgccccctacctcagtgactcgaggacggggtgaactacgcctgaggatccgatctttttccctctgccaaaaattatggggacatcatgaagccccttgagcatctgacttctggctaataaaggaaatttattttcattgcaatagtgtgttggaattttttgtgtctctcactcggcctaggtagataagtagcatggcgggttaatcattaactacaaggaacccctagtgatggagttggccactccctctctgcgcgctcgctcgctcactgaggccgggcgaccaaaggtcgcccgacgcccgggctttgcccgggcggcctcagtgagcgagcgagcgcgcag

SEQ ID NO: 138 - DNA, 1490 bp, Artificial Sequence
  Description of Artificial Sequence: Synthetic polynucleotide
ctgcgcgctcgctcgctcactgaggccgcccgggcaaagcccgggcgtcgggcgacctttggtcgcccggcctcagtgagcgagcgagcgcgcagagagggagtgtagccatgctctaggaagatcaattcaattcacgcgtcgacattgattattgactagttattaatagtaatcaattacggggtcattagttcatagcccatatatggagttccgcgttacataacttacggtaaatggcccgcctggctgaccgcccaacgacccccgcccattgacgtcaataatgacgtatgttcccatagtaacgccaatagggactttccattgacgtcaatgggtggagtatttacggtaaactgcccacttggcagtacatcaagtgtatcatatgccaagtacgccccctattgacgtcaatgacggtaaatggcccgcctggcattatgcccagtacatgaccttatgggactttcctacttggcagtacatctacgtattagtcatcgctattaccatgtcgaggccacgttctgcttcactctccccatctcccccccctccccacccccaattttgtatttatttattttttaattattttgtgcagcgatgggggcggggggggggggcgcgcgccaggcggggcggggcggggcgaggggcggggcggggcgaggcggagaggtgcggcggcagccaatcagagcggcgcgctccgaaagtttccttttatggcgaggcggcggcggcggcggccctataaaaagcgaagcgcgcggcgggcgggagcaagcttgaactgaaaaaccagaaagttaactggtaagtttagtctttttgtcttttatttcaggtcccggatccggtggtggtgcaaatcaaagaactgctcctcagtggatgttgcctttacttctaggcctgtacggaagtgttacttctgctctaaaagctgcggaattgtacccgcggccgatccaccggtaccgagctgtgctgggcggggggcggcgggccctcccgcagaacaccatgcgctcttcggaagcaggtcctcactttaattcctgtgacctgggattaaagtgaggacctgcttctgaggagcgccttgacagcagccatgggagggccgccccctacctcagtgactcgaggacggggtgaactacgcctgaggatccgatctttttccctctgccaaaaattatggggacatcatgaagccccttgagcatctgacttctggctaataaaggaaatttattttcattgcaatagtgtgttggaattttttgtgtctctcactcggcctaggtagataagtagcatggcgggttaatcattaactacaaggaacccctagtgatggagttggccactccctctctgcgcgctcgctcgctcactgaggccgggcgaccaaaggtcgcccgacgcccgggctttgcccgggcggcctcagtgagcgagcgagcgcgcag

SEQ ID NO: 139 - DNA, 1584 bp, Artificial Sequence
  Description of Artificial Sequence: Synthetic polynucleotide
ctgcgcgctcgctcgctcactgaggccgcccgggcaaagcccgggcgtcgggcgacctttggtcgcccggcctcagtgagcgagcgagcgcgcagagagggagtgtagccatgctctaggaagatcaattcaattcacgcgtcgacattgattattgactagttattaatagtaatcaattacggggtcattagttcatagcccatatatggagttccgcgttacataacttacggtaaatggcccgcctggctgaccgcccaacgacccccgcccattgacgtcaataatgacgtatgttcccatagtaacgccaatagggactttccattgacgtcaatgggtggagtatttacggtaaactgcccacttggcagtacatcaagtgtatcatatgccaagtacgccccctattgacgtcaatgacggtaaatggcccgcctggcattatgcccagtacatgaccttatgggactttcctacttggcagtacatctacgtattagtcatcgctattaccatgtcgaggccacgttctgcttcactctccccatctcccccccctccccacccccaattttgtatttatttattttttaattattttgtgcagcgatgggggcggggggggggggcgcgcgccaggcggggcggggcggggcgaggggcggggcggggcgaggcggagaggtgcggcggcagccaatcagagcggcgcgctccgaaagtttccttttatggcgaggcggcggcggcggcggccctataaaaagcgaagcgcgcggcgggcgggagcaagcttgaactgaaaaaccagaaagttaactggtaagtttagtctttttgtcttttatttcaggtcccggatccggtggtggtgcaaatcaaagaactgctcctcagtggatgttgcctttacttctaggcctgtacggaagtgttacttctgctctaaaagctgcggaattgtacccgcggccgatccaccggtgaagcaaagaaggggcagagggagcccgtgagctgagtgggccagggactgggagaaggagtgaggaggcagggccggcatgcctctgctgctggccagaggcaatgtgactgctggtaccgtctgcacctgtcactagtgccagcagtcacattgcctttggccgtgtagtgctacccagcgctggctgcctcctcagcattgcaattcctctcccatctgggcaccagtcagctaccctggtgggaatctgggtagccctcgaggacggggtgaactacgcctgaggatccgatctttttccctctgccaaaaattatggggacatcatgaagccccttgagcatctgacttctggctaataaaggaaatttattttcattgcaatagtgtgttggaattttttgtgtctctcactcggcctaggtagataagtagcatggcgggttaatcattaactacaaggaacccctagtgatggagttggccactccctctctgcgcgctcgctcgctcactgaggccgggcgaccaaaggtcgcccgacgcccgggctttgcccgggcggcctcagtgagcgagcgagcgcgcag

SEQ ID NO: 140 - DNA, 1491 bp, Artificial Sequence
  Description of Artificial Sequence: Synthetic polynucleotide
ctgcgcgctcgctcgctcactgaggccgcccgggcaaagcccgggcgtcgggcgacctttggtcgcccggcctcagtgagcgagcgagcgcgcagagagggagtgtagccatgctctaggaagatcaattcaattcacgcgtcgacattgattattgactagttattaatagtaatcaattacggggtcattagttcatagcccatatatggagttccgcgttacataacttacggtaaatggcccgcctggctgaccgcccaacgacccccgcccattgacgtcaataatgacgtatgttcccatagtaacgccaatagggactttccattgacgtcaatgggtggagtatttacggtaaactgcccacttggcagtacatcaagtgtatcatatgccaagtacgccccctattgacgtcaatgacggtaaatggcccgcctggcattatgcccagtacatgaccttatgggactttcctacttggcagtacatctacgtattagtcatcgctattaccatgtcgaggccacgttctgcttcactctccccatctcccccccctccccacccccaattttgtatttatttattttttaattattttgtgcagcgatgggggcggggggggggggcgcgcgccaggcggggcggggcggggcgaggggcggggcggggcgaggcggagaggtgcggcggcagccaatcagagcggcgcgctccgaaagtttccttttatggcgaggcggcggcggcggcggccctataaaaagcgaagcgcgcggcgggcgggagcaagcttgaactgaaaaaccagaaagttaactggtaagtttagtctttttgtcttttatttcaggtcccggatccggtggtggtgcaaatcaaagaactgctcctcagtggatgttgcctttacttctaggcctgtacggaagtgttacttctgctctaaaagctgcggaattgtacccgcggccgatccaccggtaccgagctggtgctgggcggggggcggcgggccctcccgcagaacaccatgcgctcttcggaagcaggtcctcactttaatccctgtgacctgggattaaagtgaggacctgcttctgtggagcgccttgacagcagccatgggagggccgccccctacctcagtgactcgaggacggggtgaactacgcctgaggatccgatctttttccctctgccaaaaattatggggacatcatgaagccccttgagcatctgacttctggctaataaaggaaatttattttcattgcaatagtgtgttggaattttttgtgtctctcactcggcctaggtagataagtagcatggcgggttaatcattaactacaaggaacccctagtgatggagttggccactccctctctgcgcgctcgctcgctcactgaggccgggcgaccaaaggtcgcccgacgcccgggctttgcccgggcggcctcagtgagcgagcgagcgcgcag

SEQ ID NO: 141 - DNA, 1490 bp, Artificial Sequence
  Description of Artificial Sequence: Synthetic polynucleotide
ctgcgcgctcgctcgctcactgaggccgcccgggcaaagcccgggcgtcgggcgacctttggtcgcccggcctcagtgagcgagcgagcgcgcagagagggagtgtagccatgctctaggaagatcaattcaattcacgcgtcgacattgattattgactagttattaatagtaatcaattacggggtcattagttcatagcccatatatggagttccgcgttacataacttacggtaaatggcccgcctggctgaccgcccaacgacccccgcccattgacgtcaataatgacgtatgttcccatagtaacgccaatagggactttccattgacgtcaatgggtggagtatttacggtaaactgcccacttggcagtacatcaagtgtatcatatgccaagtacgccccctattgacgtcaatgacggtaaatggcccgcctggcattatgcccagtacatgaccttatgggactttcctacttggcagtacatctacgtattagtcatcgctattaccatgtcgaggccacgttctgcttcactctccccatctcccccccctccccacccccaattttgtatttatttattttttaattattttgtgcagcgatgggggcggggggggggggcgcgcgccaggcggggcggggcggggcgaggggcggggcggggcgaggcggagaggtgcggcggcagccaatcagagcggcgcgctccgaaagtttccttttatggcgaggcggcggcggcggcggccctataaaaagcgaagcgcgcggcgggcgggagcaagcttgaactgaaaaaccagaaagttaactggtaagtttagtctttttgtcttttatttcaggtcccggatccggtggtggtgcaaatcaaagaactgctcctcagtggatgttgcctttacttctaggcctgtacggaagtgttacttctgctctaaaagctgcggaattgtacccgcggccgatccaccggtaccgagctgtgctgggcggggggcggcgggccctcccgcagaacaccatgcgctcttcggaagcaggtcctgactttaatccctgtgacctgggattaaagtgaggacctgcttctgtggagcgccttgacagcagccatgggagggccgccccctacctcagtgactcgaggacggggtgaactacgcctgaggatccgatctttttccctctgccaaaaattatggggacatcatgaagccccttgagcatctgacttctggctaataaaggaaatttattttcattgcaatagtgtgttggaattttttgtgtctctcactcggcctaggtagataagtagcatggcgggttaatcattaactacaaggaacccctagtgatggagttggccactccctctctgcgcgctcgctcgctcactgaggccgggcgaccaaaggtcgcccgacgcccgggctttgcccgggcggcctcagtgagcgagcgagcgcgcag

SEQ ID NO: 142 - DNA, 1490 bp, Artificial Sequence
  Description of Artificial Sequence: Synthetic polynucleotide
ctgcgcgctcgctcgctcactgaggccgcccgggcaaagcccgggcgtcgggcgacctttggtcgcccggcctcagtgagcgagcgagcgcgcagagagggagtgtagccatgctctaggaagatcaattcaattcacgcgtcgacattgattattgactagttattaatagtaatcaattacggggtcattagttcatagcccatatatggagttccgcgttacataacttacggtaaatggcccgcctggctgaccgcccaacgacccccgcccattgacgtcaataatgacgtatgttcccatagtaacgccaatagggactttccattgacgtcaatgggtggagtatttacggtaaactgcccacttggcagtacatcaagtgtatcatatgccaagtacgccccctattgacgtcaatgacggtaaatggcccgcctggcattatgcccagtacatgaccttatgggactttcctacttggcagtacatctacgtattagtcatcgctattaccatgtcgaggccacgttctgcttcactctccccatctcccccccctccccacccccaattttgtatttatttattttttaattattttgtgcagcgatgggggcggggggggggggcgcgcgccaggcggggcggggcggggcgaggggcggggcggggcgaggcggagaggtgcggcggcagccaatcagagcggcgcgctccgaaagtttccttttatggcgaggcggcggcggcggcggccctataaaaagcgaagcgcgcggcgggcgggagcaagcttgaactgaaaaaccagaaagttaactggtaagtttagtctttttgtcttttatttcaggtcccggatccggtggtggtgcaaatcaaagaactgctcctcagtggatgttgcctttacttctaggcctgtacggaagtgttacttctgctctaaaagctgcggaattgtacccgcggccgatccaccggtaccgagctgtgctgggcggggggcggcgggccctcccgcagaacaccatgcgctcttcggaagcaggtcctcactttaatgcctgtgacctgggattaaagtgaggacctgcttctgaggagcgccttgacagcagccatgggagggccgccccctacctcagtgactcgaggacggggtgaactacgcctgaggatccgatctttttccctctgccaaaaattatggggacatcatgaagccccttgagcatctgacttctggctaataaaggaaatttattttcattgcaatagtgtgttggaattttttgtgtctctcactcggcctaggtagataagtagcatggcgggttaatcattaactacaaggaacccctagtgatggagttggccactccctctctgcgcgctcgctcgctcactgaggccgggcgaccaaaggtcgcccgacgcccgggctttgcccgggcggcctcagtgagcgagcgagcgcgcag

SEQ ID NO: 143 - DNA, 1490 bp, Artificial Sequence
  Description of Artificial Sequence: Synthetic polynucleotide
ctgcgcgctcgctcgctcactgaggccgcccgggcaaagcccgggcgtcgggcgacctttggtcgcccggcctcagtgagcgagcgagcgcgcagagagggagtgtagccatgctctaggaagatcaattcaattcacgcgtcgacattgattattgactagttattaatagtaatcaattacggggtcattagttcatagcccatatatggagttccgcgttacataacttacggtaaatggcccgcctggctgaccgcccaacgacccccgcccattgacgtcaataatgacgtatgttcccatagtaacgccaatagggactttccattgacgtcaatgggtggagtatttacggtaaactgcccacttggcagtacatcaagtgtatcatatgccaagtacgccccctattgacgtcaatgacggtaaatggcccgcctggcattatgcccagtacatgaccttatgggactttcctacttggcagtacatctacgtattagtcatcgctattaccatgtcgaggccacgttctgcttcactctccccatctcccccccctccccacccccaattttgtatttatttattttttaattattttgtgcagcgatgggggcggggggggggggcgcgcgccaggcggggcggggcggggcgaggggcggggcggggcgaggcggagaggtgcggcggcagccaatcagagcggcgcgctccgaaagtttccttttatggcgaggcggcggcggcggcggccctataaaaagcgaagcgcgcggcgggcgggagcaagcttgaactgaaaaaccagaaagttaactggtaagtttagtctttttgtcttttatttcaggtcccggatccggtggtggtgcaaatcaaagaactgctcctcagtggatgttgcctttacttctaggcctgtacggaagtgttacttctgctctaaaagctgcggaattgtacccgcggccgatccaccggtaccgagctgtgctgggcggggggcggcgggccctcccgcagaacaccatgcgctcttcggaagcaggtcctcactttaatccctgtgatttgggattaaagtgaggacctgcttctgaggagcgccttgacagcagccatgggagggccgccccctacctcagtgactcgaggacggggtgaactacgcctgaggatccgatctttttccctctgccaaaaattatggggacatcatgaagccccttgagcatctgacttctggctaataaaggaaatttattttcattgcaatagtgtgttggaattttttgtgtctctcactcggcctaggtagataagtagcatggcgggttaatcattaactacaaggaacccctagtgatggagttggccactccctctctgcgcgctcgctcgctcactgaggccgggcgaccaaaggtcgcccgacgcccgggctttgcccgggcggcctcagtgagcgagcgagcgcgcag

SEQ ID NO: 144 - DNA, 1584 bp, Artificial Sequence
  Description of Artificial Sequence: Synthetic polynucleotide
ctgcgcgctcgctcgctcactgaggccgcccgggcaaagcccgggcgtcgggcgacctttggtcgcccggcctcagtgagcgagcgagcgcgcagagagggagtgtagccatgctctaggaagatcaattcaattcacgcgtcgacattgattattgactagttattaatagtaatcaattacggggtcattagttcatagcccatatatggagttccgcgttacataacttacggtaaatggcccgcctggctgaccgcccaacgacccccgcccattgacgtcaataatgacgtatgttcccatagtaacgccaatagggactttccattgacgtcaatgggtggagtatttacggtaaactgcccacttggcagtacatcaagtgtatcatatgccaagtacgccccctattgacgtcaatgacggtaaatggcccgcctggcattatgcccagtacatgaccttatgggactttcctacttggcagtacatctacgtattagtcatcgctattaccatgtcgaggccacgttctgcttcactctccccatctcccccccctccccacccccaattttgtatttatttattttttaattattttgtgcagcgatgggggcggggggggggggcgcgcgccaggcggggcggggcggggcgaggggcggggcggggcgaggcggagaggtgcggcggcagccaatcagagcggcgcgctccgaaagtttccttttatggcgaggcggcggcggcggcggccctataaaaagcgaagcgcgcggcgggcgggagcaagcttgaactgaaaaaccagaaagttaactggtaagtttagtctttttgtcttttatttcaggtcccggatccggtggtggtgcaaatcaaagaactgctcctcagtggatgttgcctttacttctaggcctgtacggaagtgttacttctgctctaaaagctgcggaattgtacccgcggccgatccaccggtgaagcaaagaaggggcagagggagcccgtgagctgagtgggccagggactgggagaaggagtgaggaggcagggccggcatgcctctgctgctggccagaccccttaactcatttgttcccgtctgcacctgtcactagtaacagatgagttaaggggtttggccgtgtagtgctacccagcgctggctgcctcctcagcattgcaattcctctcccatctgggcaccagtcagctaccctggtgggaatctgggtagccctcgaggacggggtgaactacgcctgaggatccgatctttttccctctgccaaaaattatggggacatcatgaagccccttgagcatctgacttctggctaataaaggaaatttattttcattgcaatagtgtgttggaattttttgtgtctctcactcggcctaggtagataagtagcatggcgggttaatcattaactacaaggaacccctagtgatggagttggccactccctctctgcgcgctcgctcgctcactgaggccgggcgaccaaaggtcgcccgacgcccgggctttgcccgggcggcctcagtgagcgagcgagcgcgcag

SEQ ID NO: 145 - DNA, 1406 bp, Artificial Sequence; identical to SEQ ID NO: 128
  Description of Artificial Sequence: Synthetic polynucleotide

SEQ ID NO: 146 - DNA, 1406 bp, Artificial Sequence; identical to SEQ ID NO: 129
  Description of Artificial Sequence: Synthetic polynucleotide

SEQ ID NO: 147 - DNA, 2052 bp, Artificial Sequence
  Description of Artificial Sequence: Synthetic polynucleotide
ctgcgcgctcgctcgctcactgaggccgcccgggcaaagcccgggcgtcgggcgacctttggtcgcccggcctcagtgagcgagcgagcgcgcagagagggagtgtagccatgctctaggaagatcaattcaattcacgcgtcgacattgattattgactagttattaatagtaatcaattacggggtcattagttcatagcccatatatggagttccgcgttacataacttacggtaaatggcccgcctggctgaccgcccaacgacccccgcccattgacgtcaataatgacgtatgttcccatagtaacgccaatagggactttccattgacgtcaatgggtggagtatttacggtaaactgcccacttggcagtacatcaagtgtatcatatgccaagtacgccccctattgacgtcaatgacggtaaatggcccgcctggcattatgcccagtacatgaccttatgggactttcctacttggcagtacatctacgtattagtcatcgctattaccatgtcgaggccacgttctgcttcactctccccatctcccccccctccccacccccaattttgtatttatttattttttaattattttgtgcagcgatgggggcggggggggggggcgcgcgccaggcggggcggggcggggcgaggggcggggcggggcgaggcggagaggtgcggcggcagccaatcagagcggcgcgctccgaaagtttccttttatggcgaggcggcggcggcggcggccctataaaaagcgaagcgcgcggcgggcgggagcaagcttgaactgaaaaaccagaaagttaactggtaagtttagtctttttgtcttttatttcaggtcccggatccggtggtggtgcaaatcaaagaactgctcctcagtggatgttgcctttacttctaggcctgtacggaagtgttacttctgctctaaaagctgcggaattgtacccgcggccgatccaccggtcaccatggtgagcaagggcgaggaggataacatggccatcatcaaggagttcatgcgcttcaaggtgcacatggagggctccgtgaacggccacgagttcgagatcgagggcgagggcgagggccgcccctacgagggcacccagaccgccaagctgaaggtgaccaagggtggccccctgcccttcgcctgggacatcctgtcccctcagttcatgtacggctccaaggcctacgtgaagcaccccgccgacatccccgactacttgaagctgtccttccccgagggcttcaagtgggagcgcgtgatgaacttcgaggacggcggcgtggtgaccgtgacccaggactcctccctgcaggacggcgagttcatctacaaggtgaagctgcgcggcaccaacttcccctccgacggccccgtaatgcagaagaagaccatgggctgggaggcctcctccgagcggatgtaccccgaggacggcgccctgaagggcgagatcaagcagaggctgaagctgaaggacggcggccactacgacgctgaggtcaagaccacctacaaggccaagaagcccgtgcagctgcccggcgcctacaacgtcaacatcaagttggacatcacctcccacaacgaggactacaccatcgtggaacagtacgaacgcgccgagggccgccactccaccggcggcatggacgagctgtacaagtccggactcagatagtctcgaggacggggtgaactacgcctgaggatccgatctttttccctctgccaaaaattatggggacatcatgaagccccttgagcatctgacttctggctaataaaggaaatttattttcattgcaatagtgtgttggaattttttgtgtctctcactcggcctaggtagataagtagcatggcgggttaatcattaactacaaggaacccctagtgatggagttggccactccctctctgcgcgctcgctcgctcactgaggccgggcgaccaaaggtcgcccgacgcccgggctttgcccgggcggcctcagtgagcgagcgagcgcgcag